European Patent Application EP 4 201 416 A1, published June 28, 2023. Title: 一种细菌在制备免疫检查点抑制剂的增效剂中的应用. Applicant: 中山大学肿瘤防治中心（中山大学附属肿瘤医院、中山大学肿瘤研究所）. The sequence listing filed with the application follows.

SEQUENCE LISTING (1 sequence)

SEQ ID NO: 1 - DNA, 1487 bp, Alistipes finegoldii
  source 1..1487: mol_type = genomic DNA
agagtttgatcctggctcaggatgaacgctagcggcaggcttaacacatgcaagtcgaggggcagcggggagtagcaatactccgccggcgaccggcgcacgggtgcgtaacgcgtatgcaacctacctttaacaggggcataacactgagaaattggtactaattccccataacattcgagaaggcatcttcttgggttaaaaactccggtggttaaagatgggcatgcgttgtattagctagttggtgaggtaacggctcaccaaggcaacgatacatagggggactgagaggttaaccccccacattggtactgagacacggaccaaactcctacgggaggcagcagtgaggaatattggtcaatggacgcaagtctgaaccagccatgccgcgtgcaggaagacggctctatgagttgtaaactgcttttgtactagggtaaacgcttttacgtgtaggagcctgaaagtatagtacgaataaggatcggctaactccgtgccagcagccgcggtaatacggaggatccaagcgttatccggatttattgggtttaaagggtgcgtaggcggtttgataagttagaggtgaaataccggggctcaactccggaactgcctctaatactgttgaactagagagtagttgcggtaggcggaatgtatggtgtagcggtgaaatgcttagagatcatacagaacaccgattgcgaaggcagcttaccaaactatatctgacgttgaggcacgaaagcgtggggagcaaacaggattagataccctggtagtccacgcagtaaacgatgataactcgttgtcggcgatacacagtcggtgactaagcgaaagcgataagttatccacctggggagtacgttcgcaagaatgaaactcaaaggaattgacgggggcccgcacaagcggaggaacatgtggtttaattcgatgatacgcgaggaaccttacccgggcttgaaagttagtgacgattctggaaacaggatttcccttcggggcacgaaactaggtgctgcatggttgtcgtcagctcgtgccgtgaggtgtcgggttaagtcccataacgagcgcaacccctaccgttagttgccatcaggtcaagctgggcactctggcgggactgccggtgtaagccgagaggaaggtggggatgacgtcaaatcagcacggcccttacgtccggggctacacacgtgttacaatggtaggtacagagggccgctaccccgcgaggggatgccaatctcgaaagcctatctcagttcggatcggaggctgaaacccgcctccgtgaagttggattcgctagtaatcgcgcatcagccatggcgcggtgaatacgttcccgggccttgtacacaccgcccgtcaagccatggaagctgggggtgcctgaagttcgtgaccgcaaggagcgacctagggcaaaaccggtgactggggctaagtcgtaacaaggtaaccaa